European Patent Application EP 4 130 033 A1, published February 8, 2023. Title: Epitope region-bridging biparatopic antibody, and method for producing the same. Applicant: NATIONAL INSTITUTES OF BIOMEDICAL INNOVATION, HEALTH AND NUTRITION. The sequence listing filed with the application follows.

SEQUENCE LISTING (40 sequences)

SEQ ID NO: 1 - protein, 122 aa, artificial sequence
  TR45_VH
EVQLQQSGPEMEKPGASVKISCKASGYSFTGYNMNWVKQSIGKSLEWIGKIDPYYGGTDYNLRFKDKATLTVDKSSSTAYMHLSRLTSEDSAVYYCAREPNYGSNDWYFDVWGAGTTVTVSS

SEQ ID NO: 2 - protein, 119 aa, Artificial Sequence
  TR92_VH
KVQLQQSGAELVKPGASVKLSCKASGYTFTESIIHWVKQRSGQGLEWIGWFYPGSDNINYNEKFKDKATLTADKSSSTVYMELTRLTSEDSAVYFCASHEGPYVYFDYWGQGTTLTVSS

SEQ ID NO: 3 - protein, 118 aa, Artificial Sequence
  TR94_VH
QVQLQQSGAELARPGTSVKLSCKASGYTFTSYWMQWVKQTPGQGLEWIGAIYPGDGDSRYIQKFKGKATLTADKSSSTAYMQLSSLASEDSAVYYCARDGNYYAMDYWGQGTSVTVSS

SEQ ID NO: 4 - protein, 114 aa, Artificial Sequence
  TR96_VH
EVQLQQSGAELVKPGASVKLSCTPSGFNIKDTYMHWVKQRPEQGLEWIGRIDPANGYTEYDPKFQDKATITADTSSNTAYLQLSSLTSEDTAVYYCADTQLYYWGQGTTLTVSS

SEQ ID NO: 5 - protein, 117 aa, Artificial Sequence
  TR109_VH
QVQLKESGPGLVAPSQSLSITCTVSGFSLTVYGVNWVRQPPGKGLEWLGMIWGDGSTAYNSALKSRLTITKDNSKTQVFLKMNSLQTDDTARYYCARDGRRYALDYWGQGTSVTVSS

SEQ ID NO: 6 - protein, 108 aa, Artificial Sequence
  TR45_VL
DIQVTQTTSSLSASLGDRVTISCRASQDIDNYLNWYQQRPDGTVKLLIYYTSILHSGVPSRFSGSGSRTDFSLTISSLEEEDFATYFCQQGNTLPWTFGGGTKLEFKR

SEQ ID NO: 7 - protein, 108 aa, Artificial Sequence
  TR92_VL
DIVMTQSHKFMSTSVGDRVSITCKASQDVSTAVAWYQQKPGQSPKLLIYWTSTRHTGVPDRFTGSGSGTDYTLTISSVQAEDLALYYCQHHYSTPYTFGGGTKLEIQR

SEQ ID NO: 8 - protein, 109 aa, Artificial Sequence
  TR94_VL
QIVLTQSPAIMSASLGERVTITCTASSSVSSTYLHWYQQKPGSSPKLWIYSTSNLASGVPARFSGSGSGTSYSLTISSMEAEDAATYYCHQYHRSPPTFGAGTKLELKR

SEQ ID NO: 9 - protein, 109 aa, Artificial Sequence
  TR96_VL
QIVLTQSPAIMSASLGERVTMTCTASSSVSSTYLHWYQQKPGSSPKLWIYSTSNLASGVPARFSGSGSGTSYSLTISNMEAEDAATYYCHQYHRSPLTFGAGTKLELKR

SEQ ID NO: 10 - protein, 112 aa, Artificial Sequence
  TR109_VL
DIVLTQSPTSLAVSLGQRATISCRASESVDSYGDSFLHWYQQKPGQPPILLIYRASNLDSGIPARFSGSGSRTDFTLTINPVEADDVATYYCQQSNEDPYTFGGGTKLEINR

SEQ ID NO: 11 - protein, 5 aa, Artificial Sequence
  TR45_VH_CDR1
GYNMN

SEQ ID NO: 12 - protein, 17 aa, Artificial Sequence
  TR45_VH_CDR2
KIDPYYGGTDYNLRFKD

SEQ ID NO: 13 - protein, 13 aa, Artificial Sequence
  TR45_VH_CDR3
EPNYGSNDWYFDV

SEQ ID NO: 14 - protein, 5 aa, Artificial Sequence
  TR92_VH_CDR1
ESIIH

SEQ ID NO: 15 - protein, 17 aa, Artificial Sequence
  TR92_VH_CDR2
WFYPGSDNINYNEKFKD

SEQ ID NO: 16 - protein, 10 aa, Artificial Sequence
  TR92_VH_CDR3
HEGPYVYFDY

SEQ ID NO: 17 - protein, 5 aa, Artificial Sequence
  TR94_VH_CDR1
SYWMQ

SEQ ID NO: 18 - protein, 17 aa, Artificial Sequence
  TR94_VH_CDR2
AIYPGDGDSRYIQKFKG

SEQ ID NO: 19 - protein, 9 aa, Artificial Sequence
  TR94_VH_CDR3
DGNYYAMDY

SEQ ID NO: 20 - protein, 5 aa, Artificial Sequence
  TR96_VH_CDR1
DTYMH

SEQ ID NO: 21 - protein, 17 aa, Artificial Sequence
  TR96_VH_CDR2
RIDPANGYTEYDPKFQD

SEQ ID NO: 22 - protein, 5 aa, Artificial Sequence
  TR96_VH_CDR3
TQLYY

SEQ ID NO: 23 - protein, 5 aa, Artificial Sequence
  TR109_VH_CDR1
VYGVN

SEQ ID NO: 24 - protein, 16 aa, Artificial Sequence
  TR109_VH_CDR2
MIWGDGSTAYNSALKS

SEQ ID NO: 25 - protein, 9 aa, Artificial Sequence
  TR109_VH_CDR3
DGRRYALDY

SEQ ID NO: 26 - protein, 11 aa, Artificial Sequence
  TR45_VL_CDR1
RASQDIDNYLN

SEQ ID NO: 27 - protein, 7 aa, Artificial Sequence
  TR45_VL_CDR2
YTSILHS

SEQ ID NO: 28 - protein, 9 aa, Artificial Sequence
  TR45_VL_CDR3
QQGNTLPWT

SEQ ID NO: 29 - protein, 11 aa, Artificial Sequence
  TR92_VL_CDR1
KASQDVSTAVA

SEQ ID NO: 30 - protein, 8 aa, Artificial Sequence
  TR92_VL_CDR2
YWTSTRHT

SEQ ID NO: 31 - protein, 9 aa, Artificial Sequence
  TR92_VL_CDR3
QHHYSTPYT

SEQ ID NO: 32 - protein, 12 aa, Artificial Sequence
  TR94_VL_CDR1
TASSSVSSTYLH

SEQ ID NO: 33 - protein, 7 aa, Artificial Sequence
  TR94_VL_CDR2
STSNLAS

SEQ ID NO: 34 - protein, 9 aa, Artificial Sequence
  TR94_VL_CDR3
HQYHRSPPT

SEQ ID NO: 35 - protein, 12 aa, Artificial Sequence
  TR96_VL_CDR1
TASSSVSSTYLH

SEQ ID NO: 36 - protein, 7 aa, Artificial Sequence
  TR96_VL_CDR2
STSNLAS

SEQ ID NO: 37 - protein, 9 aa, Artificial Sequence
  TR96_VL_CDR3
HQYHRSPLT

SEQ ID NO: 38 - protein, 15 aa, Artificial Sequence
  TR109_VL_CDR1
RASESVDSYGDSFLH

SEQ ID NO: 39 - protein, 7 aa, Artificial Sequence
  TR109_VL_CDR2
RASNLDS

SEQ ID NO: 40 - protein, 9 aa, Artificial Sequence
  TR109_VL_CDR3
QQSNEDPYT